European Patent Application EP 4 650 778 A1, published November 19, 2025. Title: ABCG1磷酸化位点作为肿瘤生物标记物的用途. Applicant: 复旦大学附属肿瘤医院. The sequence listing filed with the application follows.

SEQUENCE LISTING (16 sequences)

SEQ ID NO: 1 - protein, 14 aa, artificial sequence
  MOD_RES 12: note = Phosphorylation
CPEGPWWRKKGYKT

SEQ ID NO: 2 - protein, 16 aa, artificial sequence
  MOD_RES 7: note = Phosphorylation
RKKGYKTLLKGISGKC

SEQ ID NO: 3 - protein, 14 aa, artificial sequence
  MOD_RES 5: note = Phosphorylation
CMGPSGAGKSTLMN

SEQ ID NO: 4 - protein, 14 aa, artificial sequence
  MOD_RES 10: note = Phosphorylation
CMGPSGAGKSTLMN

SEQ ID NO: 5 - protein, 14 aa, artificial sequence
  MOD_RES 10: note = Phosphorylation
CQGGRSIICTIHQP

SEQ ID NO: 6 - protein, 14 aa, artificial sequence
  MOD_RES 4: note = Phosphorylation
HQPSAKLFELFDQC

SEQ ID NO: 7 - protein, 13 aa, artificial sequence
  MOD_RES 10: note = Phosphorylation
CGNEAKKVLSNSG

SEQ ID NO: 8 - protein, 14 aa, artificial sequence
  MOD_RES 2: note = Phosphorylation
AYFVLRYKIRAERC

SEQ ID NO: 9 - protein, 14 aa, artificial sequence
CPEGPWWRKKGYKT

SEQ ID NO: 10 - protein, 16 aa, artificial sequence
RKKGYKTLLKGISGKC

SEQ ID NO: 11 - protein, 14 aa, artificial sequence
CMGPSGAGKSTLMN

SEQ ID NO: 12 - protein, 14 aa, artificial sequence
CMGPSGAGKSTLMN

SEQ ID NO: 13 - protein, 14 aa, artificial sequence
CQGGRSIICTIHQP

SEQ ID NO: 14 - protein, 14 aa, artificial sequence
HQPSAKLFELFDQC

SEQ ID NO: 15 - protein, 13 aa, artificial sequence
CGNEAKKVLSNSG

SEQ ID NO: 16 - protein, 14 aa, artificial sequence
AYFVLRYKIRAERC